European Patent Application EP 4 293 038 A1, published December 20, 2023. Title: EPITOPE PEPTIDE AND ANTIBODY FOR PREVENTING AND TREATING EB VIRUS INFECTION AND RELATED DISEASE. Applicant: XIAMEN UNIVERSITY; SUN YAT-SEN UNIVERSITY CANCER CENTER (SUN YAT-SEN UNIVERSITY CANCER HOSPITAL, SUN YAT-SEN UNIVERSITY CANCER INSTITUTE); SUN YAT-SEN UNIVERSITY. Application PCT/CN2022/074985. The sequence listing filed with the application follows.

SEQUENCE LISTING (33 sequences)

SEQ ID NO: 1 - protein, 111 aa, Artificial Sequence
  3A3 VH
QSVKESGGRLVTPGTPLTLTCTVSGFSLSSYAMSWVRQAPGKGLEYIGVIYASGSTYYASWAKGRFTISRTATTVDLKITSPTTEDTATYFCGRGVSTNMWGPGTLVTVSS

SEQ ID NO: 2 - protein, 112 aa, Artificial Sequence
  3A3 VL
DLVMTQTPSSVSAAVGGTVTIKCQASQSLGGGLAWYQQKPGQRPKLLIYSASTLESGVPSRFRGSGSGTEFTLTISDLECADAATYYCQSAYGPTSNGLFNAFGGGTKVVIK

SEQ ID NO: 3 - protein, 8 aa, Artificial Sequence
  3A3 CDR-H1
GFSLSSYA

SEQ ID NO: 4 - protein, 7 aa, Artificial Sequence
  3A3 CDR-H2
IYASGST

SEQ ID NO: 5 - protein, 8 aa, Artificial Sequence
  3A3 CDR-H3
GRGVSTNM

SEQ ID NO: 6 - protein, 6 aa, Artificial Sequence
  3A3 CDR-L1
QSLGGG

SEQ ID NO: 7 - protein, 3 aa, Artificial Sequence
  3A3 CDR-L2
SAS

SEQ ID NO: 8 - protein, 14 aa, Artificial Sequence
  3A3 CDR-L3
QSAYGPTSNGLFNA

SEQ ID NO: 9 - protein, 119 aa, Artificial Sequence
  3A5 VH
QSVKESGGRLVTPGTPLTLTCTVSGFSLSSYEMGWVRQAPGEGLEWIGTISTGGSSYYASWAKGRFTISRTSTTVDLKMTSLTTADTATYFCARGYGGYGIGAGYFNIWGPGTLVTVSS

SEQ ID NO: 10 - protein, 110 aa, Artificial Sequence
  3A5 VL
ALVMTQTPSSVSEPVGGTVTIKCQASQSISSYLAWYQRKPGQRPKLLIYGTSTLASGVPSRFIGSGSGTDYTLTISDLECDDAATYYCQQGFSTSNVYNSFGGGTKVDIK

SEQ ID NO: 11 - protein, 8 aa, Artificial Sequence
  3A5 CDR-H1
GFSLSSYE

SEQ ID NO: 12 - protein, 7 aa, Artificial Sequence
  3A5 CDR-H2
ISTGGSS

SEQ ID NO: 13 - protein, 16 aa, Artificial Sequence
  3A5 CDR-H3
ARGYGGYGIGAGYFNI

SEQ ID NO: 14 - protein, 6 aa, Artificial Sequence
  3A5 CDR-L1
QSISSY

SEQ ID NO: 15 - protein, 3 aa, Artificial Sequence
  3A5 CDR-L2
GTS

SEQ ID NO: 16 - protein, 12 aa, Artificial Sequence
  3A5 CDR-L3
QQGFSTSNVYNS

SEQ ID NO: 17 - protein, 857 aa, Artificial Sequence
  Amino acid sequence of EBV M81 strain gB protein
MTRRRVLSVVVLLAALACRLGAQTPEQPAPPATTVQPTATRQQTSFPFRVCELSSHGDLFRFSSDIQCPSFGTRENHTEGLLMVFKDNIIPYSFKVRSYTKIVTNILIYNGWYADSVTNRHEEKFSVESYETDQMDTIYQCYNAVKMTKDGLTRVYVDRDGVNITVNLKPTGGLANGVRRYASQTELYDAPGWLIWTYRTRTTVNCLITDMMAKSNSPFDFFVTTTGQTVEMSPFYDGKNTETFHERADSFHVRTNYKIVDYDNRGTNPQGERRAFLDKGTYTLSWKLENRTAYCPLQHWQTFDSTIATETGKSIHFVTDEGTSSFVTNTTVGIELPDAFKCIEEQVNKTMHEKYEAVQDRYTKGQEAITYFITSGGLLLAWLPLTPRSLATVKNLTELTTPTSSPPSSPSPPAPPAARGSTSAAVLRRRRRNAGNATTPVPPAAPGKSLGTLNNPATVQIQFAYDSLRRQINRMLGDLARAWCLEQKRQNMVLRELTKINPTTVMSSIYGKAVAAKRLGDVISVSQCVPVNQATVTLRKSMRVPGSETMCYSRPLVSFSFINDTKTYEGQLGTDNEIFLTKKMTEVCQATSQYYFQSGNEIHVYNDYHHFKTIELDGIATLQTFISLNTSLIENIDFASLELYSRDEQRASNVFDLEGIFREYNFQAQNIAGLRKDLDNAVSNGRNQFVDGLGELMDSLGSVGQSITNLVSTVGGLFSSLVSGFISFFKNPFGGMLILVLVVGVVILVISLTRRTRQMSQQPVQMLYPGIDELAQQHASGEGPGINPISKTELQAIMLALHEQNQEQKRAAQRAAGPSVASRALQAARDRFPGLRRRRYHDPETAAALLGEAETEF

SEQ ID NO: 18 - protein, 22 aa, Artificial Sequence
  EBV gB protein aa341-362
KCIEEQVNKTMHEKYEAVQDRY

SEQ ID NO: 19 - protein, 37 aa, Artificial Sequence
  EBV gB protein aa331-367
TVGIELPDAFKCIEEQVNKTMHEKYEAVQDRYTKGQE

SEQ ID NO: 20 - protein, 89 aa, Artificial Sequence
  EBV gB protein aa528-616
CVPVNQATVTLRKSMRVPGSETMCYSRPLVSFSFINDTKTYEGQLGTDNEIFLTKKMTEVCQATSQYYFQSGNEIHVYNDYHHFKTIEL

SEQ ID NO: 21 - protein, 170 aa, Artificial Sequence
  Carrier protein HBc149/mut
MDIDPYKEFGASVELLSFLPSDFFPSIRDLLDTASALYREALESPEHCSPHHTALRQAILCWGELMNLATWVGSNLEDGGGGSGGGGTGSEFGGGGSGGGGSRELVVSYVNVNMGLKIRQLLWFHISCLTFGRETVLEYLVSFGVWIRTPPAYRPQNAPILSTLPETTVV

SEQ ID NO: 22 - protein, 207 aa, Artificial Sequence
  Recombination protein gB aa331-367+ HBc149/mut
MDIDPYKEFGASVELLSFLPSDFFPSIRDLLDTASALYREALESPEHCSPHHTALRQAILCWGELMNLATWVGSNLEDGGGGSGGGGTGSETVGIELPDAFKCIEEQVNKTMHEKYEAVQDRYTKGQEFGGGGSGGGGSRELVVSYVNVNMGLKIRQLLWFHISCLTFGRETVLEYLVSFGVWIRTPPAYRPQNAPILSTLPETTVV

SEQ ID NO: 23 - protein, 857 aa, Artificial Sequence
  Amino acid sequence of EBV gB protein after amino acid substitution in Example 1
MTRRRVLSVVVLLAALACRLGAQTPEQPAPPATTVQPTATRQQTSFPFRVCELSSHGDLFRFSSDIQCPSFGTRENHTEGLLMVFKDNIIPYSFKVRSYTKIVTNILIYNGHRADSVTNRHEEKFSVESYETDQMDTIYQCYNAVKMTKDGLTRVYVDRDGVNITVNLKPTGGLANGVRRYASQTELYDAPGRVEATYRTRTTVNCLITDMMAKSNSPFDFFVTTTGQTVEMSPFYDGKNTETFHERADSFHVRTNYKIVDYDNRGTNPQGERRAFLDKGTYTLSWKLENRTAYCPLQHWQTFDSTIATETGKSIHFVTDEGTSSFVTNTTVGIELPDAFKCIEEQVNKTMHEKYEAVQDRYTKGQEAITYFITSGGLLLAWLPLTPRSLATVKNLTELTTPTSSPPSSPSPPAPPAARGSTSAAVLRRRRRNAGNATTPVPPAAPGKSLGTLNNPATVQIQFAYDSLRRQINRMLGDLARAWCLEQKRQNMVLRELTKINPTTVMSSIYGKAVAAKRLGDVISVSQCVPVNQATVTLRKSMRVPGSETMCYSRPLVSFSFINDTKTYEGQLGTDNEIFLTKKMTEVCQATSQYYFQSGNEIHVYNDYHHFKTIELDGIATLQTFISLNTSLIENIDFASLELYSRDEQRASNVFDLEGIFREYNFQAQNIAGLRKDLDNAVSNGRNQFVDGLGELMDSLGSVGQSITNLVSTVGGLFSSLVSGFISFFKNPFGGMLILVLVVGVVILVISLTRRTRQMSQQPVQMLYPGIDELAQQHASGEGPGINPISKTELQAIMLALHEQNQEQKRAAQRAAGPSVASRALQAARDRFPGLRRRRYHDPETAAALLGEAETEF

SEQ ID NO: 24 - protein, 660 aa, Artificial Sequence
  gB ectodomain in Example 1 (aa24~683)
TPEQPAPPATTVQPTATRQQTSFPFRVCELSSHGDLFRFSSDIQCPSFGTRENHTEGLLMVFKDNIIPYSFKVRSYTKIVTNILIYNGHRADSVTNRHEEKFSVESYETDQMDTIYQCYNAVKMTKDGLTRVYVDRDGVNITVNLKPTGGLANGVRRYASQTELYDAPGRVEATYRTRTTVNCLITDMMAKSNSPFDFFVTTTGQTVEMSPFYDGKNTETFHERADSFHVRTNYKIVDYDNRGTNPQGERRAFLDKGTYTLSWKLENRTAYCPLQHWQTFDSTIATETGKSIHFVTDEGTSSFVTNTTVGIELPDAFKCIEEQVNKTMHEKYEAVQDRYTKGQEAITYFITSGGLLLAWLPLTPRSLATVKNLTELTTPTSSPPSSPSPPAPPAARGSTSAAVLRRRRRNAGNATTPVPPAAPGKSLGTLNNPATVQIQFAYDSLRRQINRMLGDLARAWCLEQKRQNMVLRELTKINPTTVMSSIYGKAVAAKRLGDVISVSQCVPVNQATVTLRKSMRVPGSETMCYSRPLVSFSFINDTKTYEGQLGTDNEIFLTKKMTEVCQATSQYYFQSGNEIHVYNDYHHFKTIELDGIATLQTFISLNTSLIENIDFASLELYSRDEQRASNVFDLEGIFREYNFQAQNIAGLRKDLDNAVS

SEQ ID NO: 25 - DNA, 20 bp, Artificial Sequence
  primer
ggtcacaatctccacgctga

SEQ ID NO: 26 - DNA, 20 bp, Artificial Sequence
  primer
caacgaggctgacctgatcc

SEQ ID NO: 27 - DNA, 510 bp, Artificial Sequence
  Nucleotide sequence of carrier protein HBc149/mut
atggacattgacccttataaagaatttggagcttctgtggagttactctcttttttgccttccgacttctttccttctattcgagatctcctcgacaccgcctctgctctgtatcgggaggccttagagtctccggaacattgttcacctcaccatacggcactcaggcaagctattctgtgttggggtgagttgatgaatctagccacctgggtgggaagtaatttggaagatggtggaggtggttctggaggtggtggtactggatccgaattcggtggtggaggttcaggaggaggtggttccagggaactagtagtcagctatgtcaacgttaatatgggcctaaaaatcagacaactattgtggtttcacatttcctgtcttacttttgggagagaaactgttcttgaatatttggtgtcttttggagtgtggattcgcactcctcctgcatatagaccacaaaatgcccctatcttatcaacacttccggaaactactgttgtt

SEQ ID NO: 28 - DNA, 351 bp, Artificial Sequence
  VH nucleotide sequence of control antibody 1E12
cagtcagtgaaggagtccgggggtcgcctggtcacgcctgggacacccctgacactcacctgcaccgtctctggaatcgacctcagtacctatgtaatgacttgggtccgccaggctccagggaaggggctggaatgcatcggaatcattggttatggtggtagcacatactacgcgagctgggcgacaggccgattcaccatctccaaaacctcgaccacggtggatctgagaatgaccagtctgacaaccgaggacacggccacctatttctgtgccagaggtgttagtagtaatctttataggggaatgaatttgtggggccaaggcaccctggtcaccgtctcttca

SEQ ID NO: 29 - DNA, 333 bp, Artificial Sequence
  VL nucleotide sequence of control antibody 1E12
gccctcgtgatgacccagactccatctcccgtgtctgcagctgtgggaggcacagtcagcatcagttgccagtccagtccgagtgtttatagtaattacttatcctggtatcagcagaaaccagggcagcctcccaagctcctgatctacgaaacatccaaactggaatctggggtcccatcgcggttcagcggcagtggatctgggacacagttcactctcaccatcagcggcgtgcaatgtgacgatgctgccacttactactgtgcaggcggttatagtggtattagtgatacgtttgctttcggcggagggaccaaggtggacatcaaa

SEQ ID NO: 30 - protein, 330 aa, Artificial Sequence [sequence omitted]

SEQ ID NO: 31 - protein, 107 aa, Artificial Sequence
  Human light chain constant region sequence
RTVAAPSVFIFPPSDEQLKSGTASVVCLLNNFYPREAKVQWKVDSALQSGNSQESVTEQDSKDSTYSLSSTLTLSKADYEKHKVYACEVTHQGLSSPVTKSFNRGEC

SEQ ID NO: 32 - protein, 121 aa, Artificial Sequence
  Control antibody VRC01-VH
QVQLVQSGGQMKKPGESMRISCRASGYEFIDCTLNWIRLAPGKRPEWMGWLKPRGGAVNYARPLQGRVTMTRDVYSDTAFLELRSLTVDDTAVYFCTRGKNCDYNWDFEHWGRGTPVIVSS

SEQ ID NO: 33 - protein, 104 aa, Artificial Sequence
  Control antibody VRC01-VL
EIVLTQSPGTLSLSPGETAIISCRTSQYGSLAWYQQRPGQAPRLVIYSGSTRAAGIPDRFSGSRWGPDYNLTISNLESGDFGVYYCQQYEFFGQGTKVQVDIKR